European Patent Application EP 4 786 488 A1, published August 5, 2026. Title: 经修饰的铁蛋白、交联铁蛋白及其制备方法和应用. Applicant: 上海尚泽涌致生物科技合伙企业（有限合伙）. The sequence listing filed with the application follows.

SEQUENCE LISTING (7 sequences)

SEQ ID NO: 1 - protein, 174 aa, synthetic construct
SSQIRQNYSTDVEAAVNSLVNLYLQASYTYLSLGFYFDRDDVALEGVSHFFRELAEEKREGYERLLKMQNQRGGRALFQDIKKPAEDEWGKTPDAMKAAMALEKKLNQALLDLHALGSARTDPHLCDFLETHFLDEEVKLIKKMGDHLTNLHRLGGPEAGLGEYLFERLTLKHD

SEQ ID NO: 2 - protein, 183 aa, synthetic construct
MTTASTSQVRQNYHQDSEAAINRQINLELYASYVYLSMSYYFDRDDVALKNFAKYFLHQSHEEREHAEKLMKLQNQRGGRIFLQDIKKPDCDDWESGLNAMECALHLEKNVNQSLLELHKLATDKNDPHLCDFIETHYLNEQVKAIKELGDHVTNLRKMGAPESGLAEYLFDKHTLGDSDNES

SEQ ID NO: 3 - protein, 171 aa, synthetic construct
MAESQCRQNYHQESEAGINRQINMELYACYTYQSMAYYFDRDDVALPGFSKFFKNSSDEEREHAEKLMKYQNKRGGRVVLQDIKKPDRDEWGTGLDAMQVALQLEKTVNQSLLDLHKVADSHQDAQMCDFLETHYLEEQVNAIKEISDHITQLKRVGSGLGEYEYDRRLDS

SEQ ID NO: 4 - protein, 158 aa, synthetic construct
MKGDKKVIQHLNKILGNELIAINQYFLHSRMWNDWGLKRLGAHEYHESIDEMKHADKLIERILFLEGLPNLQDLGKLLIGENTQEMLQCDLNLELKATKDLREAIVHCEQVHDYVSRDLLKDILESEEEHIDYLETQLGLIQKVGLENYLQSHMHEDD

SEQ ID NO: 5 - protein, 165 aa, synthetic construct
MLKPEMIEKLNEQMNLELYSSLLYQQMSAWCSYHTFEGAAAFLRRHAQEEMTHMQRLFDYLTDTGNLPRINTVESPFAEYSSLDELFQETYKHEQLITQKINELAHAAMTNQDYPTFNFLQWYVSEQHEEEKLFKSIIDKLSLAGKSGEGLYFIDKELSTLDTQN

SEQ ID NO: 6 - protein, 177 aa, synthetic construct
MTTASTSQVRQNYHQDSEAAINRQINLELYASYVYLSMSYYFDRDDVALKNFAKYFLHQSHEEREHAEKLMKLQNQRGGRIFLQDIKKPDCDDWESGLNAMECALHLEKNVNQSLLELHKLATDKNDPHLCDFIETHYLIKELGDHVTNLRKMGAPESGLAEYLFDKHTLGDSDNES

SEQ ID NO: 7 - protein, 177 aa, synthetic construct
MTTASTSQVRQNYHQDSEAAINRQINLELYASYVYLSMSYYFDRDDVALKNFAKYFLHQSHEEREHAEKLMKLQNQRGGRIFLQDIKKPDCDDWESGLNAMECALHLEKNVNQSLLELHKLATDKNDPHLCDFIETHYLIKELGCHVTNLRKMGAPESGLAEYLFDKHTLGDSDNES